European Patent Application EP 4 563 159 A1, published June 4, 2025. Title: Mucosal vaccination via an IgA feedback loop. Applicant: Forschungszentrum Borstel, Leibniz Lungenzentrum. The sequence listing filed with the application follows.

SEQUENCE LISTING (47 sequences)

SEQ ID NO: 1 - protein, 20 aa, Severe acute respiratory syndrome-related coronavirus type 2
FPLQSYGFQPTNGVGYQPYR

SEQ ID NO: 2 - protein, 20 aa, Severe acute respiratory syndrome-related coronavirus type 2
FPLKSYSFRPTYGVGHQPYR

SEQ ID NO: 3 - protein, 50 aa, Streptococcus pyogenes
YYALSDAKEEEPRYKALRGENQDLREKERKYQDKIKKLEEKEKNLEKKSC

SEQ ID NO: 4 - protein, 18 aa, synthetic construct
  VARIANT 1..3: note = each X independently represents an arbitrary amino acid residue other than cysteine
  VARIANT 6: note = each X independently represents an arbitrary amino acid residue other than cysteine
  VARIANT 8: note = each X independently represents an arbitrary amino acid residue other than cysteine
  VARIANT 9..10: note = each X independently represents an arbitrary amino acid residue other than cysteine or is deleted
  VARIANT 12..13: note = each X independently represents an arbitrary amino acid residue other than cysteine
  VARIANT 16..18: note = each X independently represents an arbitrary amino acid residue other than cysteine
XXXCLXYXXXGXXVCXXX

SEQ ID NO: 5 - protein, 16 aa, synthetic construct
HMRCLHYKGRRVCFLL

SEQ ID NO: 6 - protein, 16 aa, synthetic construct
QMRCLSYKGRRVCLWL

SEQ ID NO: 7 - protein, 16 aa, synthetic construct
HKRCLHYRGRMVCFLI

SEQ ID NO: 8 - protein, 16 aa, synthetic construct
KRLCLQYKGSKVCFRL

SEQ ID NO: 9 - protein, 16 aa, synthetic construct
RMRCLTYRGRRVCLEL

SEQ ID NO: 10 - protein, 16 aa, synthetic construct
SMRCLQYRGSRVCLTL

SEQ ID NO: 11 - protein, 16 aa, synthetic construct
QKRCLKYKGSRVCFFL

SEQ ID NO: 12 - protein, 16 aa, synthetic construct
HLRCLRYKGTRVCFSL

SEQ ID NO: 13 - protein, 16 aa, synthetic construct
HVRCLSYKGREVCVQL

SEQ ID NO: 14 - protein, 16 aa, synthetic construct
PRMCLHYKGRRVCIPY

SEQ ID NO: 15 - protein, 16 aa, synthetic construct
HVRCLRYRGKNVCFLL

SEQ ID NO: 16 - protein, 16 aa, synthetic construct
SDVCLRYRGRPVCFQV

SEQ ID NO: 17 - protein, 16 aa, synthetic construct
RDVCLRYRGRPVCFQV

SEQ ID NO: 18 - protein, 16 aa, synthetic construct
HDVCLRYRGRPVCFQV

SEQ ID NO: 19 - protein, 16 aa, synthetic construct
SMVCLRYRGRPVCFQV

SEQ ID NO: 20 - protein, 16 aa, synthetic construct
SAVCLRYRGRPVCFQV

SEQ ID NO: 21 - protein, 16 aa, synthetic construct
SDVCLNYRGRPVCFQV

SEQ ID NO: 22 - protein, 16 aa, synthetic construct
SDVCLHYRGRPVCFQV

SEQ ID NO: 23 - protein, 16 aa, synthetic construct
SDVCLAYRGRPVCFQV

SEQ ID NO: 24 - protein, 16 aa, synthetic construct
SDVCLRYRGRPVCFRV

SEQ ID NO: 25 - protein, 16 aa, synthetic construct
SDVCLRYRGRPVCFLV

SEQ ID NO: 26 - protein, 16 aa, synthetic construct
SDVCLRYRGRPVCFAV

SEQ ID NO: 27 - protein, 16 aa, synthetic construct
SDVCLRYRGRPVCFQL

SEQ ID NO: 28 - protein, 16 aa, synthetic construct
SDVCLRYRGRPVCFQA

SEQ ID NO: 29 - protein, 16 aa, synthetic construct
HMVCLAYRGRPVCFAL

SEQ ID NO: 30 - protein, 16 aa, synthetic construct
HMVCLSYRGRPVCFSL

SEQ ID NO: 31 - protein, 16 aa, synthetic construct
HQVCLSYRGRPVCFST

SEQ ID NO: 32 - protein, 16 aa, synthetic construct
  VARIANT 1..3: note = each X independently represents an arbitrary amino acid residue other than cysteine
  VARIANT 6: note = each X independently represents an arbitrary amino acid residue other than cysteine
  VARIANT 8: note = each X independently represents an arbitrary amino acid residue other than cysteine
  VARIANT 10..11: note = each X independently represents an arbitrary amino acid residue other than cysteine
  VARIANT 14..15: note = each X independently represents an arbitrary amino acid residue other than cysteine
  VARIANT 16: note = T or L
XXXCLXYXGXXVCXXX

SEQ ID NO: 33 - protein, 16 aa, synthetic construct
  VARIANT 1: note = H, K, Q, G or P
  VARIANT 2: note = M, S, F, V or Q
  VARIANT 3: note = V or R, A, W
  VARIANT 6: note = A or S
  VARIANT 15: note = P, F, A, G or S
  VARIANT 16: note = T or L
XXXCLXYRGRXVCFXX

SEQ ID NO: 34 - protein, 16 aa, synthetic construct
  VARIANT 1: note = H, K or P
  VARIANT 2: note = M, S, F or Q
  VARIANT 3: note = V or R
  VARIANT 6: note = A or S
  VARIANT 11: note = P or S
  VARIANT 15: note = P or S
XXXCLXYRGRXVCFXT

SEQ ID NO: 35 - protein, 16 aa, synthetic construct
KMVCLAYRGRPVCFPT

SEQ ID NO: 36 - protein, 16 aa, synthetic construct
HSVCLAYRGRPVCFPT

SEQ ID NO: 37 - protein, 16 aa, synthetic construct
KFRCLSYRGRSVCFST

SEQ ID NO: 38 - protein, 16 aa, synthetic construct
PQVCLAYRGRPVCFST

SEQ ID NO: 39 - protein, 16 aa, synthetic construct
KMACLAYRGRPGCFFT

SEQ ID NO: 40 - protein, 16 aa, synthetic construct
QSWCLAYRGRPVCFRT

SEQ ID NO: 41 - protein, 16 aa, synthetic construct
HMVCLAYRGRPVCFPT

SEQ ID NO: 42 - protein, 16 aa, synthetic construct
HVVCLAYRGRPVCFPT

SEQ ID NO: 43 - protein, 16 aa, synthetic construct
HMVCLSYRGRPVCFST

SEQ ID NO: 44 - protein, 16 aa, synthetic construct
KMVCLSYRGRPVCFST

SEQ ID NO: 45 - protein, 16 aa, synthetic construct
GMRCLSYRGRPVCFST

SEQ ID NO: 46 - protein, 16 aa, synthetic construct
HSRCLAYRGRPVCFAL

SEQ ID NO: 47 - protein, 16 aa, synthetic construct
HQVCLAYRGRPVCFGL